European Patent Specification EP 4 267 115 B1, published January 28, 2026. Title: Nanostructured delivery system for tumor treatment. Applicant: Universitaetsklinikum Jena. Application EP 20217124.5. The sequence listing filed with the application follows.

SEQUENCE LISTING (4 sequences)

SEQ ID NO: 1 - DNA, 20 bp, Artificial Sequence
  Primer
gtccagtcattggctttgca

SEQ ID NO: 2 - DNA, 22 bp, Artificial Sequence
  Primer
caacccaacgagagtccttagg

SEQ ID NO: 3 - DNA, 22 bp, Artificial Sequence
  Primer
agaaacgattgcagggtttcac

SEQ ID NO: 4 - DNA, 22 bp, Artificial Sequence
  Primer
ccgagtgaagatccccttttta